European Patent Application EP 4 506 455 A1, published February 12, 2025. Title: Cell suitable for genetic engineering, cell engineering, and cell therapy and method of producing the same. Applicant: Logomix, Inc. The sequence listing filed with the application follows.

SEQUENCE LISTING (73 sequences)

SEQ ID NO: 1 - RNA, 20 nt, Synthetic construct
  source 1..20: mol_type = other RNA
cttcatctccgtcggctacg

SEQ ID NO: 2 - RNA, 20 nt, synthetic construct
  source 1..20: mol_type = other RNA
atgatggaaaactcgatggg

SEQ ID NO: 3 - RNA, 20 nt, synthetic construct
  source 1..20: mol_type = other RNA
tggaatccggtataggcgcc

SEQ ID NO: 4 - RNA, 20 nt, synthetic construct
  source 1..20: mol_type = other RNA
tgagtgacccgataaaactc

SEQ ID NO: 5 - RNA, 20 nt, synthetic construct
  source 1..20: mol_type = other RNA
tcttaaaaacttctatatcg

SEQ ID NO: 6 - RNA, 20 nt, synthetic construct
  source 1..20: mol_type = other RNA
gtgcaactcccgaataggct

SEQ ID NO: 7 - RNA, 20 nt, synthetic construct
  source 1..20: mol_type = other RNA
tgggccttatcatccgtcaa

SEQ ID NO: 8 - RNA, 20 nt, synthetic construct
  source 1..20: mol_type = other RNA
tgggtctgtcgagcacaagg

SEQ ID NO: 9 - RNA, 20 nt, synthetic construct
  source 1..20: mol_type = other RNA
ggtcaaatgccttgtactcg

SEQ ID NO: 10 - RNA, 20 nt, synthetic construct
  source 1..20: mol_type = other RNA
gggagggccggtaccgttga

SEQ ID NO: 11 - RNA, 20 nt, synthetic construct
  source 1..20: mol_type = other RNA
atagctaacgtcactattgc

SEQ ID NO: 12 - RNA, 20 nt, synthetic construct
  source 1..20: mol_type = other RNA
cgttctcagcgcgggcacta

SEQ ID NO: 13 - RNA, 20 nt, synthetic construct
  source 1..20: mol_type = other RNA
gccgctgccgctctacgctt

SEQ ID NO: 14 - RNA, 20 nt, synthetic construct
  source 1..20: mol_type = other RNA
cagaaagggtaagcgcacag

SEQ ID NO: 15 - RNA, 20 nt, synthetic construct
  source 1..20: mol_type = other RNA
ggcgcaacgcgatcgcgtaa

SEQ ID NO: 16 - RNA, 20 nt, synthetic construct
  source 1..20: mol_type = other RNA
gacgccagtgcattcgacga

SEQ ID NO: 17 - RNA, 20 nt, synthetic construct
  source 1..20: mol_type = other RNA
ggcgcaacgcgatcgcgtaa

SEQ ID NO: 18 - DNA, 20 bp, synthetic construct
  source 1..20: mol_type = other DNA
cctcaccttcccctcttttc

SEQ ID NO: 19 - DNA, 20 bp, unidentified
  source 1..20: mol_type = other DNA
accttcccctgtgacttgtg

SEQ ID NO: 20 - DNA, 20 bp, synthetic construct
  source 1..20: mol_type = other DNA
ctcaccttcccttcctttcc

SEQ ID NO: 21 - DNA, 20 bp, synthetic construct
  source 1..20: mol_type = other DNA
accttcccctgtgatttgtg

SEQ ID NO: 22 - DNA, 20 bp, synthetic construct
  source 1..20: mol_type = other DNA
ccaccaccctgtctttgact

SEQ ID NO: 23 - DNA, 20 bp, synthetic construct
  source 1..20: mol_type = other DNA
tgtcaccccttccttacctg

SEQ ID NO: 24 - DNA, 20 bp, synthetic construct
  source 1..20: mol_type = other DNA
gaggcagaaaggcacacata

SEQ ID NO: 25 - DNA, 20 bp, synthetic construct
  source 1..20: mol_type = other DNA
agcctctccttcccattctt

SEQ ID NO: 26 - DNA, 22 bp, synthetic construct
  source 1..22: mol_type = other DNA
tccatcaacctctcatagcaaa

SEQ ID NO: 27 - DNA, 21 bp, synthetic construct
  source 1..21: mol_type = other DNA
acttctggaaattccttttgg

SEQ ID NO: 28 - DNA, 18 bp, synthetic construct
  source 1..18: mol_type = other DNA
gatggcccatgtgtggat

SEQ ID NO: 29 - DNA, 20 bp, synthetic construct
  source 1..20: mol_type = other DNA
ttatcccaggtgcctgtgtc

SEQ ID NO: 30 - DNA, 20 bp, synthetic construct
  source 1..20: mol_type = other DNA
ttcccacttacagccagacc

SEQ ID NO: 31 - DNA, 20 bp, synthetic construct
  source 1..20: mol_type = other DNA
tacgggaggtagccagtgtt

SEQ ID NO: 32 - DNA, 21 bp, synthetic construct
  source 1..21: mol_type = other DNA
tgggaagtggtcaggagataa

SEQ ID NO: 33 - DNA, 18 bp, synthetic construct
  source 1..18: mol_type = other DNA
ggccttccatctgttgct

SEQ ID NO: 34 - DNA, 18 bp, synthetic construct
  source 1..18: mol_type = other DNA
gacatcggcaaggtgtgg

SEQ ID NO: 35 - DNA, 19 bp, synthetic construct
  source 1..19: mol_type = other DNA
gtggtggagtgaacggaga

SEQ ID NO: 36 - DNA, 21 bp, synthetic construct
  source 1..21: mol_type = other DNA
tgggaagtggtcaggagataa

SEQ ID NO: 37 - DNA, 24 bp, synthetic construct
  source 1..24: mol_type = other DNA
tgtaatcttctctgtcgctacttc

SEQ ID NO: 38 - DNA, 20 bp, synthetic construct
  source 1..20: mol_type = other DNA
tgcaccagattgttttgtgt

SEQ ID NO: 39 - DNA, 19 bp, synthetic construct
  source 1..19: mol_type = other DNA
gtggtggagtgaacggaga

SEQ ID NO: 40 - DNA, 20 bp, synthetic construct
  source 1..20: mol_type = other DNA
ccaccttagcctcctcctct

SEQ ID NO: 41 - DNA, 21 bp, synthetic construct
  source 1..21: mol_type = other DNA
aaagcatatttgggcactctg

SEQ ID NO: 42 - DNA, 20 bp, synthetic construct
  source 1..20: mol_type = other DNA
agacaagttcaccccaccag

SEQ ID NO: 43 - DNA, 20 bp, synthetic construct
  source 1..20: mol_type = other DNA
tcacctccatgtgccttaca

SEQ ID NO: 44 - DNA, 20 bp, synthetic construct
  source 1..20: mol_type = other DNA
acagagagaagggcacagga

SEQ ID NO: 45 - DNA, 20 bp, synthetic construct
  source 1..20: mol_type = other DNA
catcagcagaagggaggaag

SEQ ID NO: 46 - DNA, 20 bp, synthetic construct
  source 1..20: mol_type = other DNA
aacatgcaaaggggattctg

SEQ ID NO: 47 - DNA, 20 bp, synthetic construct
  source 1..20: mol_type = other DNA
tggaagtggcttttggtttc

SEQ ID NO: 48 - DNA, 20 bp, synthetic construct
  source 1..20: mol_type = other DNA
tggatttcatgcctcacaaa

SEQ ID NO: 49 - DNA, 20 bp, synthetic construct
  source 1..20: mol_type = other DNA
ttcctcttgtctccccagaa

SEQ ID NO: 50 - DNA, 20 bp, synthetic construct
  source 1..20: mol_type = other DNA
caccatcacccttcttccac

SEQ ID NO: 51 - DNA, 20 bp, synthetic construct
  source 1..20: mol_type = other DNA
tgcttcctcttcccagctaa

SEQ ID NO: 52 - DNA, 20 bp, synthetic construct
  source 1..20: mol_type = other DNA
caccatcacccttcttccac

SEQ ID NO: 53 - DNA, 20 bp, synthetic construct
  source 1..20: mol_type = other DNA
tgcttcctcttcccagctaa

SEQ ID NO: 54 - DNA, 20 bp, synthetic construct
  source 1..20: mol_type = other DNA
gcagagagtgggaccaagag

SEQ ID NO: 55 - DNA, 20 bp, synthetic construct
  source 1..20: mol_type = other DNA
tgctaattctggggagatgg

SEQ ID NO: 56 - DNA, 20 bp, synthetic construct
  source 1..20: mol_type = other DNA
tccatcagggtcttctggtc

SEQ ID NO: 57 - DNA, 20 bp, synthetic construct
  source 1..20: mol_type = other DNA
tttttaaccggctctggatg

SEQ ID NO: 58 - DNA, 20 bp, synthetic construct
  source 1..20: mol_type = other DNA
gagagcccttagctggtgtg

SEQ ID NO: 59 - DNA, 20 bp, synthetic construct
  source 1..20: mol_type = other DNA
gtgcagtttgtccacccttt

SEQ ID NO: 60 - DNA, 21 bp, synthetic construct
  source 1..21: mol_type = other DNA
tgggaagtggtcaggagataa

SEQ ID NO: 61 - DNA, 40 bp, synthetic construct
  source 1..40: mol_type = other DNA
gtctgggtaagggccagggcccccgagagtagcaggagga

SEQ ID NO: 62 - DNA, 20 bp, synthetic construct
  source 1..20: mol_type = other DNA
acgtagggtccttcatcctg

SEQ ID NO: 63 - DNA, 19 bp, synthetic construct
  source 1..19: mol_type = other DNA
gtggtggagtgaacggaga

SEQ ID NO: 64 - DNA, 21 bp, synthetic construct
  source 1..21: mol_type = other DNA
tgggaagtggtcaggagataa

SEQ ID NO: 65 - DNA, 20 bp, synthetic construct
  source 1..20: mol_type = other DNA
agacaactgccaaggacacc

SEQ ID NO: 66 - DNA, 19 bp, synthetic construct
  source 1..19: mol_type = other DNA
gtggtggagtgaacggaga

SEQ ID NO: 67 - DNA, 20 bp, synthetic construct
  source 1..20: mol_type = other DNA
ccctgtgtgagtccagaaca

SEQ ID NO: 68 - DNA, 21 bp, synthetic construct
  source 1..21: mol_type = other DNA
tgggaagtggtcaggagataa

SEQ ID NO: 69 - DNA, 20 bp, synthetic construct
  source 1..20: mol_type = other DNA
ccctgtgtgagtccagaaca

SEQ ID NO: 70 - DNA, 19 bp, synthetic construct
  source 1..19: mol_type = other DNA
gtggtggagtgaacggaga

SEQ ID NO: 71 - DNA, 20 bp, synthetic construct
  source 1..20: mol_type = other DNA
ccctgtgtgagtccagaaca

SEQ ID NO: 72 - protein, 361 aa, synthetic construct
MAVMAPRTLLLLLSGALALTQTWAGSHSLKYFHTSVSRPGRGEPRFISVGYVDDTQFVRFDNDAASPRMVPRAPWMEQEGSEYWDRETRSARDTAQIFRVNLRTLRGYYNQSEAGSHTLQWMHGCELGPDRRFLRGYEQFAYDGKDYLTLNEDLRSWTAVDTAAQISEQKSNDASEAEHQRAYLEDTCVEWLHKYLEKGKETLLHLEPPKTHVTHHPISDHEATLRCWALGFYPAEITLTWQQDGEGHTQDTELVETRPAGDGTFQKWAAVVVPSGEEQRYTCHVQHEGLPEPVTLRWKPASQPTIPIVGIIAGLVLLGSVVSGAVVAAVIWRKKSSGGKGGSYSKAEWSDSAQGSESHSL

SEQ ID NO: 73 - protein, 14 aa, synthetic construct
AVMAPRTLLLLLSG